European Patent Application EP 4 578 871 A1, published July 2, 2025. Title: IL2 variants and protein complex comprising thereof. Applicant: MUSTBIO Co., Ltd. The sequence listing filed with the application follows.

SEQUENCE LISTING (83 sequences)

SEQ ID NO: 1 - protein, 133 aa, synthetic construct
APTSSSTKKTQLQLEHLLLDLQMILNGINNYKNPELTAMLTKKFYMPKKATELKHLQCLEEELKPLEEVLNLAQSKNFHLRPRDLISNINVIVLELKGSETTFMCEYADETATIVEFLNRWITFSQSIISTLT

SEQ ID NO: 2 - protein, 133 aa, synthetic construct
APTSSSTKKTQLQLEHLMSDLQMILNGINNYKNPELTAMLTKKFYMPKKATELKHLQCLEEELKPLEEVLNLAQSKNFHLRPRDLISNINVIVLELKGSETTFMCEYADETATIVEFLNRWITFSQSIISTLT

SEQ ID NO: 3 - protein, 133 aa, synthetic construct
APTSSSTKKTQLQLEHLASDLQMILNGINNYKNPELTAMLTKKFYMPKKATELKHLQCLEEELKPLEEVLNLAQSKNFHLRPRDLISNINVIVLELKGSETTFMCEYADETATIVEFLNRWITFSQSIISTLT

SEQ ID NO: 4 - protein, 133 aa, synthetic construct
APTSSSTKKTQLQLEHLRSDLQMILNGINNYKNPELTAMLTKKFYMPKKATELKHLQCLEEELKPLEEVLNLAQSKNFHLRPRDLISNINVIVLELKGSETTFMCEYADETATIVEFLNRWITFSQSIISTLT

SEQ ID NO: 5 - protein, 133 aa, synthetic construct
APTSSSTKKTQLQLEHLMLDLQMILNGINNYKNPELTAMLTKKFYMPKKATELKHLQCLEEELKPLEEVLNLAQSKNFHLRPRDLISNINVIVLELKGSETTFMCEYADETATIVEFLNRWITFSQSIISTLT

SEQ ID NO: 6 - protein, 133 aa, synthetic construct
APTSSSTKKTQLQLEHLLSDLQMILNGINNYKNPELTAMLTKKFYMPKKATELKHLQCLEEELKPLEEVLNLAQSKNFHLRPRDLISNINVIVLELKGSETTFMCEYADETATIVEFLNRWITFSQSIISTLT

SEQ ID NO: 7 - protein, 133 aa, synthetic construct
APTSSSTKKTQLQLEHLSWDLQMILNGINNYKNPELTAMLTKKFYMPKKATELKHLQCLEEELKPLEEVLNLAQSKNFHLRPRDLISNINVIVLELKGSETTFMCEYADETATIVEFLNRWITFSQSIISTLT

SEQ ID NO: 8 - protein, 133 aa, synthetic construct
APTSSSTKKTQLQLEHLFNDLQMILNGINNYKNPELTAMLTKKFYMPKKATELKHLQCLEEELKPLEEVLNLAQSKNFHLRPRDLISNINVIVLELKGSETTFMCEYADETATIVEFLNRWITFSQSIISTLT

SEQ ID NO: 9 - protein, 133 aa, synthetic construct
APTSSSTKKTQLQLEHLVIDLQMILNGINNYKNPELTAMLTKKFYMPKKATELKHLQCLEEELKPLEEVLNLAQSKNFHLRPRDLISNINVIVLELKGSETTFMCEYADETATIVEFLNRWITFSQSIISTLT

SEQ ID NO: 10 - protein, 133 aa, synthetic construct
APTSSSTKKTQLQLEHLITDLQMILNGINNYKNPELTAMLTKKFYMPKKATELKHLQCLEEELKPLEEVLNLAQSKNFHLRPRDLISNINVIVLELKGSETTFMCEYADETATIVEFLNRWITFSQSIISTLT

SEQ ID NO: 11 - protein, 133 aa, synthetic construct
APTSSSTKKTQLQLEHLQADLQMILNGINNYKNPELTAMLTKKFYMPKKATELKHLQCLEEELKPLEEVLNLAQSKNFHLRPRDLISNINVIVLELKGSETTFMCEYADETATIVEFLNRWITFSQSIISTLT

SEQ ID NO: 12 - protein, 133 aa, synthetic construct
APTSSSTKKTQLQLEHLMMDLQMILNGINNYKNPELTAMLTKKFYMPKKATELKHLQCLEEELKPLEEVLNLAQSKNFHLRPRDLISNINVIVLELKGSETTFMCEYADETATIVEFLNRWITFSQSIISTLT

SEQ ID NO: 13 - protein, 133 aa, synthetic construct
APTSSSTKKTQLQLEHLMFDLQMILNGINNYKNPELTAMLTKKFYMPKKATELKHLQCLEEELKPLEEVLNLAQSKNFHLRPRDLISNINVIVLELKGSETTFMCEYADETATIVEFLNRWITFSQSIISTLT

SEQ ID NO: 14 - protein, 133 aa, unidentified
APTSSSTKKTQLQLEHLLLDLQMILNGINNYKNPELTAMLTKKFYMPKKATELKHLQCLEEELKPLEEVLNLAQSKNFHLRPRDLISNINVIVLELKGSETTFMCEYADETATIVEFLNRWITFSTSIISTLT

SEQ ID NO: 15 - protein, 133 aa, synthetic construct
APTSSSTKKTQLQLEHLLLDLQMILNGINNYKNPELTAMLTKKFYMPKKATELKHLQCLEEELKPLEEVLNLAQSKNFHLRPRDLISNINVIVLELKGSETTFMCEYADETATIVEFLNRWITFSISIISTLT

SEQ ID NO: 16 - protein, 133 aa, synthetic construct [sequence omitted]

SEQ ID NO: 17 - protein, 133 aa, synthetic construct
APTSSSTKKTQLQLEHLLLDLQMILNGINNYKNPELTRMLTFKFYMPKKATELKHLQCLEEELKPLEEVLNLAQSKNFHLRPRDLISNINVIVLELKGSETTFMCEYADETATIVEFLNRWITFSQSIISTLT

SEQ ID NO: 18 - protein, 15 aa, synthetic construct
GGGGSGGGGSGGGGS

SEQ ID NO: 19 - protein, 232 aa, synthetic construct
EPKSCDKTHTCPPCPAPEAAGGPSVFLFPPKPKDTLMISRTPEVTCVVVDVSHEDPEVKFNWYVDGVEVHNAKTKPREEQYNSTYRVVSVLTVLHQDWLNGKEYKCKVSNKALPAPIEKTISKAKGQPREPQVYTLPPSRDELTKNQVSLWCLVKGFYPSDIAVEWESNGQPENNYKTTPPVLDSDGSFFLYSKLTVDKSRWQQGNVFSCSVMHEALHNHYTQKSLSLSPGK

SEQ ID NO: 20 - protein, 227 aa, synthetic construct
DKTHTCPPCPAPEAAGGPSVFLFPPKPKDTLMISRTPEVTCVVVDVSHEDPEVKFNWYVDGVEVHNAKTKPREEQYNSTYRVVSVLTVLHQDWLNGKEYKCKVSNKALPAPIEKTISKAKGQPREPQVYTGPPSRDELTKNQVSLSCAVKGFYPSDIAVEWESNGQPENNYKTTPPVLDSDGSFFLVSKLTVDKSRWQQGNVFSCSVMHEALHNHYTQKSLSLSPGK

SEQ ID NO: 21 - protein, 231 aa, synthetic construct
EPKSCDKTHTCPPCPAPEAAGGPSVFLFPPKPKDTLMISRTPEVTCVVVDVSHEDPEVKFNWYVDGVEVHNAKTKPREEQYNSTYRVVSVLTVLHQDWLNGKEYKCKVSNKALPAPIEKTISKAKGQPREPQVYTGPPSRDELTKNQVSLSCAVKGFYPSDIAVEWESNGQPENNYKTTPPVLDSDGSFFLVSKLTVDKSRWQQGNVFSCSVMHEALHNHYTQKSLSLSPG

SEQ ID NO: 22 - protein, 232 aa, synthetic construct
EPKSCDKTHTCPPCPAPEAAGGPSVFLFPPKPKDTLMISRTPEVTCVVVDVSHEDPEVKFNWYVDGVEVHNAKTKPREEQYNSTYRVVSVLTVLHQDWLNGKEYKCKVSNKALPAPIEKTISKAKGQPREPQVYTFPPSRDELTKNQVSLWCLVKGFYPSDIAVEWESNGQPENNYKTTPPVLDSDGSFFLYSKLTVDKSRWQQGNVFSCSVMHEALHNHYTQKSLSLSPGK

SEQ ID NO: 23 - protein, 227 aa, synthetic construct; identical to SEQ ID NO: 20

SEQ ID NO: 24 - protein, 231 aa, synthetic construct; identical to SEQ ID NO: 21

SEQ ID NO: 25 - protein, 232 aa, synthetic construct
EPKSCDKTHTCPPCPAPEAAGGPSVFLFPPKPKDTLMISRTPEVTCVVVDVSHEDPEVKFNWYVDGVEVHNAKTKPREEQYNSTYRVVSVLTVLHQDWLNGKEYKCKVSNKALPAPIEKTISKAKGQPREPQVYTWPPSRDELTKNQVSLWCLVKGFYPSDIAVEWESNGQPENNYKTTPPVLDSDGSFFLYSKLTVDKSRWQQGNVFSCSVMHEALHNHYTQKSLSLSPGK

SEQ ID NO: 26 - protein, 227 aa, synthetic construct; identical to SEQ ID NO: 20

SEQ ID NO: 27 - protein, 231 aa, synthetic construct; identical to SEQ ID NO: 21

SEQ ID NO: 28 - protein, 231 aa, unidentified
PKSCDKTHTCPPCPAPEAAGGPSVFLFPPKPKDTLMISRTPEVTCVVVDVSHEDPEVKFNWYVDGVEVHNAKTKPREEQYNSTYRVVSVLTVLHQDWLNGKEYKCKVSNKALPAPIEKTISKAKGQPREPQVYTLPPSRDELTKNQVSLWCLVKGFYPSDIAVEWESNGQPENNYKTTPPVLDSDGSFFLYSKLTVDKSRWQQGNVFSCSVMHEALHNHYTQKSLSLSPGK

SEQ ID NO: 29 - protein, 227 aa, synthetic construct
DKTHTCPPCPAPEAAGGPSVFLFPPKPKDTLMISRTPEVTCVVVDVSHEDPEVKFNWYVDGVEVHNAKTKPREEQYNSTYRVVSVLTVLHQDWLNGKEYKCKVSNKALPAPIEKTISKAKGQPREPQVYTFPPSRDELTKNQVSLSCAVKGFYPSDIAVEWESNGQPENNYKTTPPVLDSDGSFFLVSKLTVDKSRWQQGNVFSCSVMHEALHNHYTQKSLSLSPGK

SEQ ID NO: 30 - protein, 231 aa, synthetic construct
EPKSCDKTHTCPPCPAPEAAGGPSVFLFPPKPKDTLMISRTPEVTCVVVDVSHEDPEVKFNWYVDGVEVHNAKTKPREEQYNSTYRVVSVLTVLHQDWLNGKEYKCKVSNKALPAPIEKTISKAKGQPREPQVYTFPPSRDELTKNQVSLSCAVKGFYPSDIAVEWESNGQPENNYKTTPPVLDSDGSFFLVSKLTVDKSRWQQGNVFSCSVMHEALHNHYTQKSLSLSPG

SEQ ID NO: 31 - protein, 232 aa, synthetic construct
EPKSCDKTHTCPPCPAPEAAGGPSVFLFPPKPKDTLMISRTPEVTCVVVDVSHEDPEVKFNWYVDGVEVHNAKTKPREEQYNSTYRVVSVLTVLHQDWLNGKEYKCKVSNKALGAPIEKTISKAKGQPREPQVYTLPPSRDELTKNQVSLWCLVKGFYPSDIAVEWESNGQPENNYKTTPPVLDSDGSFFLYSKLTVDKSRWQQGNVFSCSVMHEALHNHYTQKSLSLSPGK

SEQ ID NO: 32 - protein, 227 aa, synthetic construct
DKTHTCPPCPAPEAAGGPSVFLFPPKPKDTLMISRTPEVTCVVVDVSHEDPEVKFNWYVDGVEVHNAKTKPREEQYNSTYRVVSVLTVLHQDWLNGKEYKCKVSNKALGAPIEKTISKAKGQPREPQVYTGPPSRDELTKNQVSLSCAVKGFYPSDIAVEWESNGQPENNYKTTPPVLDSDGSFFLVSKLTVDKSRWQQGNVFSCSVMHEALHNHYTQKSLSLSPGK

SEQ ID NO: 33 - protein, 231 aa, synthetic construct
EPKSCDKTHTCPPCPAPEAAGGPSVFLFPPKPKDTLMISRTPEVTCVVVDVSHEDPEVKFNWYVDGVEVHNAKTKPREEQYNSTYRVVSVLTVLHQDWLNGKEYKCKVSNKALGAPIEKTISKAKGQPREPQVYTGPPSRDELTKNQVSLSCAVKGFYPSDIAVEWESNGQPENNYKTTPPVLDSDGSFFLVSKLTVDKSRWQQGNVFSCSVMHEALHNHYTQKSLSLSPG

SEQ ID NO: 34 - protein, 232 aa, synthetic construct
EPKSCDKTHTCPPCPAPELLGGPSVFLFPPKPKDTLMISRTPEVTCVVVDVSHEDPEVKFNWYVDGVEVHNAKTKPREEQYASTYRVVSVLTVLHQDWLNGKEYKCKVSNKALPAPIEKTISKAKGQPREPQVYTLPPSRDELTKNQVSLWCLVKGFYPSDIAVEWESNGQPENNYKTTPPVLDSDGSFFLYSKLTVDKSRWQQGNVFSCSVMHEALHNHYTQKSLSLSPGK

SEQ ID NO: 35 - protein, 227 aa, synthetic construct
DKTHTCPPCPAPELLGGPSVFLFPPKPKDTLMISRTPEVTCVVVDVSHEDPEVKFNWYVDGVEVHNAKTKPREEQYASTYRVVSVLTVLHQDWLNGKEYKCKVSNKALPAPIEKTISKAKGQPREPQVYTGPPSRDELTKNQVSLSCAVKGFYPSDIAVEWESNGQPENNYKTTPPVLDSDGSFFLVSKLTVDKSRWQQGNVFSCSVMHEALHNHYTQKSLSLSPGK

SEQ ID NO: 36 - protein, 231 aa, synthetic construct
EPKSCDKTHTCPPCPAPELLGGPSVFLFPPKPKDTLMISRTPEVTCVVVDVSHEDPEVKFNWYVDGVEVHNAKTKPREEQYASTYRVVSVLTVLHQDWLNGKEYKCKVSNKALPAPIEKTISKAKGQPREPQVYTGPPSRDELTKNQVSLSCAVKGFYPSDIAVEWESNGQPENNYKTTPPVLDSDGSFFLVSKLTVDKSRWQQGNVFSCSVMHEALHNHYTQKSLSLSPG

SEQ ID NO: 37 - protein, 232 aa, synthetic construct
EPKSCDKTHTCPPCPAPELLGGPSVFLFPPKPKDTLMISRTPEVTCVVVDVSHEDPEVKFNWYVDGVEVHNAKTKPREEQYQSTYRVVSVLTVLHQDWLNGKEYKCKVSNKALPAPIEKTISKAKGQPREPQVYTLPPSRDELTKNQVSLWCLVKGFYPSDIAVEWESNGQPENNYKTTPPVLDSDGSFFLYSKLTVDKSRWQQGNVFSCSVMHEALHNHYTQKSLSLSPGK

SEQ ID NO: 38 - protein, 227 aa, synthetic construct
DKTHTCPPCPAPELLGGPSVFLFPPKPKDTLMISRTPEVTCVVVDVSHEDPEVKFNWYVDGVEVHNAKTKPREEQYQSTYRVVSVLTVLHQDWLNGKEYKCKVSNKALPAPIEKTISKAKGQPREPQVYTGPPSRDELTKNQVSLSCAVKGFYPSDIAVEWESNGQPENNYKTTPPVLDSDGSFFLVSKLTVDKSRWQQGNVFSCSVMHEALHNHYTQKSLSLSPGK

SEQ ID NO: 39 - protein, 231 aa, synthetic construct
EPKSCDKTHTCPPCPAPELLGGPSVFLFPPKPKDTLMISRTPEVTCVVVDVSHEDPEVKFNWYVDGVEVHNAKTKPREEQYQSTYRVVSVLTVLHQDWLNGKEYKCKVSNKALPAPIEKTISKAKGQPREPQVYTGPPSRDELTKNQVSLSCAVKGFYPSDIAVEWESNGQPENNYKTTPPVLDSDGSFFLVSKLTVDKSRWQQGNVFSCSVMHEALHNHYTQKSLSLSPG

SEQ ID NO: 40 - protein, 232 aa, synthetic construct
EPKSCDKTHTCPPCPAPELLGGPSVFLFPPKPKDTLMISRTPEVTCVVVDVSHEDPEVKFNWYVDGVEVHNAKTKPREEQYGSTYRVVSVLTVLHQDWLNGKEYKCKVSNKALPAPIEKTISKAKGQPREPQVYTLPPSRDELTKNQVSLWCLVKGFYPSDIAVEWESNGQPENNYKTTPPVLDSDGSFFLYSKLTVDKSRWQQGNVFSCSVMHEALHNHYTQKSLSLSPGK

SEQ ID NO: 41 - protein, 227 aa, synthetic construct
DKTHTCPPCPAPELLGGPSVFLFPPKPKDTLMISRTPEVTCVVVDVSHEDPEVKFNWYVDGVEVHNAKTKPREEQYGSTYRVVSVLTVLHQDWLNGKEYKCKVSNKALPAPIEKTISKAKGQPREPQVYTGPPSRDELTKNQVSLSCAVKGFYPSDIAVEWESNGQPENNYKTTPPVLDSDGSFFLVSKLTVDKSRWQQGNVFSCSVMHEALHNHYTQKSLSLSPGK

SEQ ID NO: 42 - protein, 231 aa, synthetic construct
EPKSCDKTHTCPPCPAPELLGGPSVFLFPPKPKDTLMISRTPEVTCVVVDVSHEDPEVKFNWYVDGVEVHNAKTKPREEQYGSTYRVVSVLTVLHQDWLNGKEYKCKVSNKALPAPIEKTISKAKGQPREPQVYTGPPSRDELTKNQVSLSCAVKGFYPSDIAVEWESNGQPENNYKTTPPVLDSDGSFFLVSKLTVDKSRWQQGNVFSCSVMHEALHNHYTQKSLSLSPG

SEQ ID NO: 43 - protein, 232 aa, synthetic construct
EPKSCDKTHTCPPCPAPEFEGGPSVFLFPPKPKDTLMISRTPEVTCVVVDVSHEDPEVKFNWYVDGVEVHNAKTKPREEQYNSTYRVVSVLTVLHQDWLNGKEYKCKVSNKALPASIEKTISKAKGQPREPQVYTLPPSRDELTKNQVSLWCLVKGFYPSDIAVEWESNGQPENNYKTTPPVLDSDGSFFLYSKLTVDKSRWQQGNVFSCSVMHEALHNHYTQKSLSLSPGK

SEQ ID NO: 44 - protein, 227 aa, synthetic construct
DKTHTCPPCPAPEFEGGPSVFLFPPKPKDTLMISRTPEVTCVVVDVSHEDPEVKFNWYVDGVEVHNAKTKPREEQYNSTYRVVSVLTVLHQDWLNGKEYKCKVSNKALPASIEKTISKAKGQPREPQVYTGPPSRDELTKNQVSLSCAVKGFYPSDIAVEWESNGQPENNYKTTPPVLDSDGSFFLVSKLTVDKSRWQQGNVFSCSVMHEALHNHYTQKSLSLSPGK

SEQ ID NO: 45 - protein, 231 aa, synthetic construct
EPKSCDKTHTCPPCPAPEFEGGPSVFLFPPKPKDTLMISRTPEVTCVVVDVSHEDPEVKFNWYVDGVEVHNAKTKPREEQYNSTYRVVSVLTVLHQDWLNGKEYKCKVSNKALPASIEKTISKAKGQPREPQVYTGPPSRDELTKNQVSLSCAVKGFYPSDIAVEWESNGQPENNYKTTPPVLDSDGSFFLVSKLTVDKSRWQQGNVFSCSVMHEALHNHYTQKSLSLSPG

SEQ ID NO: 46 - protein, 232 aa, synthetic construct
EPKSCDKTHTCPPCPAPEFEGGPSVFLFPPKPKDTLMISRTPEVTCVVVAVSHEDPEVKFNWYVDGVEVHNAKTKPREEQYNSTYRVVSVLTVLHQDWLNGKEYKCKVSNKALPAPIEKTISKAKGQPREPQVYTLPPSRDELTKNQVSLWCLVKGFYPSDIAVEWESNGQPENNYKTTPPVLDSDGSFFLYSKLTVDKSRWQQGNVFSCSVMHEALHNHYTQKSLSLSPGK

SEQ ID NO: 47 - protein, 227 aa, synthetic construct
DKTHTCPPCPAPEFEGGPSVFLFPPKPKDTLMISRTPEVTCVVVAVSHEDPEVKFNWYVDGVEVHNAKTKPREEQYNSTYRVVSVLTVLHQDWLNGKEYKCKVSNKALPAPIEKTISKAKGQPREPQVYTGPPSRDELTKNQVSLSCAVKGFYPSDIAVEWESNGQPENNYKTTPPVLDSDGSFFLVSKLTVDKSRWQQGNVFSCSVMHEALHNHYTQKSLSLSPGK

SEQ ID NO: 48 - protein, 231 aa, synthetic construct
EPKSCDKTHTCPPCPAPEFEGGPSVFLFPPKPKDTLMISRTPEVTCVVVAVSHEDPEVKFNWYVDGVEVHNAKTKPREEQYNSTYRVVSVLTVLHQDWLNGKEYKCKVSNKALPAPIEKTISKAKGQPREPQVYTGPPSRDELTKNQVSLSCAVKGFYPSDIAVEWESNGQPENNYKTTPPVLDSDGSFFLVSKLTVDKSRWQQGNVFSCSVMHEALHNHYTQKSLSLSPG

SEQ ID NO: 49 - protein, 218 aa, synthetic construct
EVQLLESGGGLVQPGGSLRLSCAASGFTFSSYIMMWVRQAPGKGLEWVSSIYPSGGITFYADTVKGRFTISRDNSKNTLYLQMNSLRAEDTAVYYCARIKLGTVTTVDYWGQGTLVTVSSASTKGPSVFPLAPSSKSTSGGTAALGCLVKDYFPEPVTVSWNSGALTSGVHTFPAVLQSSGLYSLSSVVTVPSSSLGTQTYICNVNHKPSNTKVDKKV

SEQ ID NO: 50 - protein, 216 aa, synthetic construct
QSALTQPASVSGSPGQSITISCTGTSSDVGGYNYVSWYQQHPGKAPKLMIYDVSNRPSGVSNRFSGSKSGNTASLTISGLQAEDEADYYCSSYTSSSTRVFGTGTKVTVLGQPKANPTVTLFPPSSEELQANKATLVCLISDFYPGAVTVAWKADGSPVKAGVETTKPSKQSNNKYAASSYLSLTPEQWKSHRSYSCQVTHEGSTVEKTVAPTECS

SEQ ID NO: 51 - protein, 219 aa, synthetic construct
EVRLLESGGGLVKPEGSLKLSCVASGFTFSDYFMSWVRQAPGKGLEWVAHIYTKSYNYATYYSGSVKGRFTISRDDSRSMVYLQMNNLRTEDTATYYCTRDGSGYPSLDFWGQGTQVTVSSASTKGPSVFPLAPSSKSTSGGTAALGCLVKDYFPEPVTVSWNSGALTSGVHTFPAVLQSSGLYSLSSVVTVPSSSLGTQTYICNVNHKPSNTKVDKKV

SEQ ID NO: 52 - protein, 216 aa, synthetic construct
YELTQPPSASVNVGETVKITCSGDQLPKYFADWFHQRSDQTILQVIYDDNKRPSGIPERISGSSSGTTATLTIRDVRAEDEGDYYCFSGYVDSDSKLYVFGSGTQLTVLGGQPKANPTVTLFPPSSEELQANKATLVCLISDFYPGAVTVAWKADGSPVKAGVETTKPSKQSNNKYAASSYLSLTPEQWKSHRSYSCQVTHEGSTVEKTVAPTECS

SEQ ID NO: 53 - protein, 218 aa, synthetic construct
QVQLVQSGVEVKKPGASVKVSCKASGYTFTNYYMYWVRQAPGQGLEWMGGINPSNGGTNFNEKFKNRVTLTTDSSTTTAYMELKSLQFDDTAVYYCARRDYRFDMGFDYWGQGTTVTVSSASTKGPSVFPLAPSSKSTSGGTAALGCLVKDYFPEPVTVSWNSGALTSGVHTFPAVLQSSGLYSLSSVVTVPSSSLGTQTYICNVNHKPSNTKVDKKV

SEQ ID NO: 54 - protein, 217 aa, synthetic construct
EIVLTQSPATLSLSPGERATLSCRASKGVSTSGYSYLHWYQQKPGQAPRLLIYLASYLESGVPARFSGSGSGTDFTLTISSLEPEDFAVYYCQHSRDLPLTFGGGTKVEIKGQPKANPTVTLFPPSSEELQANKATLVCLISDFYPGAVTVAWKADGSPVKAGVETTKPSKQSNNKYAASSYLSLTPEQWKSHRSYSCQVTHEGSTVEKTVAPTECS

SEQ ID NO: 55 - protein, 132 aa, synthetic construct
PTSSSTKKTQLQLEHLLLDLQMILNGINNYKNPKLTRMLTFKFYMPKKATELKHLQCLEEELKPLEEVLNLAQSKNFHLRPRDLISNINVIVLELKGSETTFMCEYADETATIVEFLNRWITFSQSIISTLT

SEQ ID NO: 56 - DNA, 399 bp, synthetic construct
  source 1..399: mol_type = other DNA
gctcctacctcctccagcaccaagaaaacccagctgcagttggagcatctgctgctggacctgcagatgatcctgaacggcatcaacaactacaagaaccccgagctgaccgccatgctgaccaagaaattctacatgcccaagaaggccaccgagctgaaacatctgcagtgcctggaagaggaactgaagcccctggaagaagtgctgaatctggcccagtccaagaacttccacctgaggcctcgggacctgatctccaacatcaacgtgatcgtgctggaactgaaaggctccgagacaaccttcatgtgcgagtacgccgacgagacagctaccatcgtggaatttctgaaccggtggatcaccttcagccagtccatcatctctacactgacc

SEQ ID NO: 57 - DNA, 399 bp, synthetic construct
  source 1..399: mol_type = other DNA
gctcctacctcctccagcaccaagaaaacccagctgcagttggagcatctgatgtccgacctgcagatgatcctgaacggcatcaacaactacaagaaccccgagctgaccgccatgctgaccaagaaattctacatgcccaagaaggccaccgagctgaaacatctgcagtgcctggaagaggaactgaagcccctggaagaagtgctgaatctggcccagtccaagaacttccacctgaggcctcgggacctgatctccaacatcaacgtgatcgtgctggaactgaaaggctccgagacaaccttcatgtgcgagtacgccgacgagacagctaccatcgtggaatttctgaaccggtggatcaccttcagccagtccatcatctctacactgacc

SEQ ID NO: 58 - DNA, 399 bp, synthetic construct
  source 1..399: mol_type = other DNA
gctcctacctcctccagcaccaagaaaacccagctgcagttggagcatctggcctccgacctgcagatgatcctgaacggcatcaacaactacaagaaccccgagctgaccgccatgctgaccaagaaattctacatgcccaagaaggccaccgagctgaaacatctgcagtgcctggaagaggaactgaagcccctggaagaagtgctgaatctggcccagtccaagaacttccacctgaggcctcgggacctgatctccaacatcaacgtgatcgtgctggaactgaaaggctccgagacaaccttcatgtgcgagtacgccgacgagacagctaccatcgtggaatttctgaaccggtggatcaccttcagccagtccatcatctctacactgacc

SEQ ID NO: 59 - DNA, 399 bp, synthetic construct
  source 1..399: mol_type = other DNA
gctcctacctcctccagcaccaagaaaacccagctgcagttggagcatctgcggtccgacctgcagatgatcctgaacggcatcaacaactacaagaaccccgagctgaccgccatgctgaccaagaaattctacatgcccaagaaggccaccgagctgaaacatctgcagtgcctggaagaggaactgaagcccctggaagaagtgctgaatctggcccagtccaagaacttccacctgaggcctcgggacctgatctccaacatcaacgtgatcgtgctggaactgaaaggctccgagacaaccttcatgtgcgagtacgccgacgagacagctaccatcgtggaatttctgaaccggtggatcaccttcagccagtccatcatctctacactgacc

SEQ ID NO: 60 - DNA, 399 bp, synthetic construct
  source 1..399: mol_type = other DNA
gctcctacctcctccagcaccaagaaaacccagctgcagttggagcatctgatgctggacctgcagatgatcctgaacggcatcaacaactacaagaaccccgagctgaccgccatgctgaccaagaaattctacatgcccaagaaggccaccgagctgaaacatctgcagtgcctggaagaggaactgaagcccctggaagaagtgctgaatctggcccagtccaagaacttccacctgaggcctcgggacctgatctccaacatcaacgtgatcgtgctggaactgaaaggctccgagacaaccttcatgtgcgagtacgccgacgagacagctaccatcgtggaatttctgaaccggtggatcaccttcagccagtccatcatctctacactgacc

SEQ ID NO: 61 - DNA, 399 bp, synthetic construct
  source 1..399: mol_type = other DNA
gctcctacctcctccagcaccaagaaaacccagctgcagttggagcatctgctgtccgacctgcagatgatcctgaacggcatcaacaactacaagaaccccgagctgaccgccatgctgaccaagaaattctacatgcccaagaaggccaccgagctgaaacatctgcagtgcctggaagaggaactgaagcccctggaagaagtgctgaatctggcccagtccaagaacttccacctgaggcctcgggacctgatctccaacatcaacgtgatcgtgctggaactgaaaggctccgagacaaccttcatgtgcgagtacgccgacgagacagctaccatcgtggaatttctgaaccggtggatcaccttcagccagtccatcatctctacactgacc

SEQ ID NO: 62 - DNA, 399 bp, synthetic construct
  source 1..399: mol_type = other DNA
gctcctacctcctccagcaccaagaaaacccagctgcagttggagcatctgtcctgggacctgcagatgatcctgaacggcatcaacaactacaagaaccccgagctgaccgccatgctgaccaagaaattctacatgcccaagaaggccaccgagctgaaacatctgcagtgcctggaagaggaactgaagcccctggaagaagtgctgaatctggcccagtccaagaacttccacctgaggcctcgggacctgatctccaacatcaacgtgatcgtgctggaactgaaaggctccgagacaaccttcatgtgcgagtacgccgacgagacagctaccatcgtggaatttctgaaccggtggatcaccttcagccagtccatcatctctacactgacc

SEQ ID NO: 63 - DNA, 399 bp, synthetic construct
  source 1..399: mol_type = other DNA
gctcctacctcctccagcaccaagaaaacccagctgcagttggagcatctgtttaacgacctgcagatgatcctgaacggcatcaacaactacaagaaccccgagctgaccgccatgctgaccaagaaattctacatgcccaagaaggccaccgagctgaaacatctgcagtgcctggaagaggaactgaagcccctggaagaagtgctgaatctggcccagtccaagaacttccacctgaggcctcgggacctgatctccaacatcaacgtgatcgtgctggaactgaaaggctccgagacaaccttcatgtgcgagtacgccgacgagacagctaccatcgtggaatttctgaaccggtggatcaccttcagccagtccatcatctctacactgacc

SEQ ID NO: 64 - DNA, 399 bp, synthetic construct
  source 1..399: mol_type = other DNA
gctcctacctcctccagcaccaagaaaacccagctgcagttggagcatctggtgatcgacctgcagatgatcctgaacggcatcaacaactacaagaaccccgagctgaccgccatgctgaccaagaaattctacatgcccaagaaggccaccgagctgaaacatctgcagtgcctggaagaggaactgaagcccctggaagaagtgctgaatctggcccagtccaagaacttccacctgaggcctcgggacctgatctccaacatcaacgtgatcgtgctggaactgaaaggctccgagacaaccttcatgtgcgagtacgccgacgagacagctaccatcgtggaatttctgaaccggtggatcaccttcagccagtccatcatctctacactgacc

SEQ ID NO: 65 - DNA, 399 bp, synthetic construct
  source 1..399: mol_type = other DNA
gctcctacctcctccagcaccaagaaaacccagctgcagttggagcatctgatcaccgacctgcagatgatcctgaacggcatcaacaactacaagaaccccgagctgaccgccatgctgaccaagaaattctacatgcccaagaaggccaccgagctgaaacatctgcagtgcctggaagaggaactgaagcccctggaagaagtgctgaatctggcccagtccaagaacttccacctgaggcctcgggacctgatctccaacatcaacgtgatcgtgctggaactgaaaggctccgagacaaccttcatgtgcgagtacgccgacgagacagctaccatcgtggaatttctgaaccggtggatcaccttcagccagtccatcatctctacactgacc

SEQ ID NO: 66 - DNA, 399 bp, synthetic construct
  source 1..399: mol_type = other DNA
gctcctacctcctccagcaccaagaaaacccagctgcagttggagcatctgcaggccgacctgcagatgatcctgaacggcatcaacaactacaagaaccccgagctgaccgccatgctgaccaagaaattctacatgcccaagaaggccaccgagctgaaacatctgcagtgcctggaagaggaactgaagcccctggaagaagtgctgaatctggcccagtccaagaacttccacctgaggcctcgggacctgatctccaacatcaacgtgatcgtgctggaactgaaaggctccgagacaaccttcatgtgcgagtacgccgacgagacagctaccatcgtggaatttctgaaccggtggatcaccttcagccagtccatcatctctacactgacc

SEQ ID NO: 67 - DNA, 399 bp, synthetic construct
  source 1..399: mol_type = other DNA
gctcctacctcctccagcaccaagaaaacccagctgcagttggagcatctgatgatggacctgcagatgatcctgaacggcatcaacaactacaagaaccccgagctgaccgccatgctgaccaagaaattctacatgcccaagaaggccaccgagctgaaacatctgcagtgcctggaagaggaactgaagcccctggaagaagtgctgaatctggcccagtccaagaacttccacctgaggcctcgggacctgatctccaacatcaacgtgatcgtgctggaactgaaaggctccgagacaaccttcatgtgcgagtacgccgacgagacagctaccatcgtggaatttctgaaccggtggatcaccttcagccagtccatcatctctacactgacc

SEQ ID NO: 68 - DNA, 399 bp, synthetic construct
  source 1..399: mol_type = other DNA
gctcctacctcctccagcaccaagaaaacccagctgcagttggagcatctgatgtttgacctgcagatgatcctgaacggcatcaacaactacaagaaccccgagctgaccgccatgctgaccaagaaattctacatgcccaagaaggccaccgagctgaaacatctgcagtgcctggaagaggaactgaagcccctggaagaagtgctgaatctggcccagtccaagaacttccacctgaggcctcgggacctgatctccaacatcaacgtgatcgtgctggaactgaaaggctccgagacaaccttcatgtgcgagtacgccgacgagacagctaccatcgtggaatttctgaaccggtggatcaccttcagccagtccatcatctctacactgacc

SEQ ID NO: 69 - DNA, 399 bp, synthetic construct
  source 1..399: mol_type = other DNA
gctcctacctcctccagcaccaagaaaacccagctgcagttggagcatctgctgctcgacctgcagatgatcctgaacggcatcaacaactacaagaaccccgagctgaccgccatgctgaccaagaaattctacatgcccaagaaggccaccgagctgaaacatctgcagtgcctggaagaggaactgaagcccctggaagaagtgctgaatctggcccagtccaagaacttccacctgaggcctcgggacctgatctccaacatcaacgtgatcgtgctggaactgaaaggctccgagacaaccttcatgtgcgagtacgccgacgagacagctaccatcgtggaatttctgaaccggtggatcaccttcagcacctccatcatctctacactgacc

SEQ ID NO: 70 - DNA, 399 bp, synthetic construct
  source 1..399: mol_type = other DNA
gctcctacctcctccagcaccaagaaaacccagctgcagttggagcatctgctgctggacctgcagatgatcctgaacggcatcaacaactacaagaaccccgagctgaccgccatgctgaccaagaaattctacatgcccaagaaggccaccgagctgaaacatctgcagtgcctggaagaggaactgaagcccctggaagaagtgctgaatctggcccagtccaagaacttccacctgaggcctcgggacctgatctccaacatcaacgtgatcgtgctggaactgaaaggctccgagacaaccttcatgtgcgagtacgccgacgagacagctaccatcgtggaatttctgaaccggtggatcaccttctccatctccatcatctctaccctgacc

SEQ ID NO: 71 - DNA, 399 bp, synthetic construct
  source 1..399: mol_type = other DNA
gcacctacttcaagttctacaaagaaaacacagctacaactggagcatttactgctggatttacagatgattttgaatggaattaataattacaagaatcccaaactcaccaggatgctcacatttaagttttacatgcccaagaaggccacagaactgaaacatcttcagtgtctagaagaagaactcaaacctctggaggaagtgctaaatttagctcaaagcaaaaactttcacttaagacccagggacttaatcagcaatatcaacgtaatagttctggaactaaagggatctgaaacaacattcatgtgtgaatatgctgatgagacagcaaccattgtagaatttctgaacagatggattaccttttgtcaaagcatcatctcaacactgact

SEQ ID NO: 72 - DNA, 399 bp, synthetic construct
  source 1..399: mol_type = other DNA
gcccctaccagcagcagcaccaagaaaacccagctgcaactggaacacctcctgctggacctgcagatgatcctgaacggcatcaacaactacaagaaccccgagctgacccggatgctgaccttcaagttctacatgcccaagaaggccaccgagctgaagcacctccagtgcctggaagaggaactgaagcccctggaagaagtgctgaatctggcccagagcaagaacttccacctgaggccaagggacctgatcagcaacatcaacgtgatcgtgctggaactgaaaggcagcgagacaaccttcatgtgcgagtacgccgacgagacagccaccatcgtcgagtttctgaaccggtggatcaccttcagccagagcatcatcagcacactgaca

SEQ ID NO: 73 - DNA, 45 bp, synthetic construct
  source 1..45: mol_type = other DNA
ggtggcggaggatctggcggtggtggttctggcggaggcggatct

SEQ ID NO: 74 - DNA, 696 bp, synthetic construct
  source 1..696: mol_type = other DNA
gaacccaagtcctgcgacaagacccacacctgtcctccatgtcctgctccagaagctgctggcggtccctccgttttcctgtttccacctaagcctaaggacaccctgatgatctctcggacccctgaagtgacctgcgtggtggtggatgtgtctcacgaggacccagaagtgaagtttaattggtacgtggacggcgtggaagtgcacaacgccaagaccaagcctagagaggaacagtacaactccacctacagagtggtgtccgtgctgaccgtgctgcaccaggattggctgaacggcaaagagtacaagtgcaaggtgtccaacaaggccctgcctgctcctatcgaaaagaccatctccaaggctaagggccagcctcgggaacctcaggtttacacactgcctccatctcgggacgagctgaccaagaatcaggtgtccctgtggtgcctggttaagggcttctacccttccgacattgccgtggaatgggagtctaacggccagccagagaacaactacaagacaacccctcctgtgctggactccgacggctcattcttcctgtactccaagctgacagtggacaagtctcggtggcagcagggcaacgtgttctcctgttctgtgatgcacgaggccctgcacaaccactacacacagaagtccctgtctctgagccccggcaaa

SEQ ID NO: 75 - DNA, 681 bp, synthetic construct
  source 1..681: mol_type = other DNA
gataagacccacacctgtcctccatgtcctgctccagaagctgctggcggaccctctgtgttcctgtttcctccaaagcctaaggacaccctgatgatctctcggacccctgaagtgacctgcgtggtggtggatgtgtctcacgaggacccagaagtgaagtttaattggtacgtggacggcgtggaagtgcacaacgccaagaccaagcctagagaggaacagtacaactccacctacagagtggtgtccgtgctgaccgtgctgcaccaggattggctgaatggcaaagagtacaagtgcaaggtgtccaacaaggccctgcctgctcctatcgaaaagaccatctccaaggctaagggccagcctcgggaacctcaggtttacacaggacctccatctcgggacgagctgacaaagaaccaggtgtccctgtcttgcgccgtgaagggcttctacccttccgacattgccgtggaatgggagtccaatggccagcctgagaacaattacaagaccacacctcctgtgctggactccgacggctcattcttcctggtgtccaagctgacagtggacaagtccagatggcagcagggcaacgtgttctcctgctctgtgatgcacgaggccctgcacaaccactacacacagaagtccctgagcctgtctcctggcaag

SEQ ID NO: 76 - DNA, 693 bp, synthetic construct
  source 1..693: mol_type = other DNA
gaacccaagtcctgcgataagacccacacctgtcctccatgtcctgctccagaagctgctggcggaccctctgtgttcctgtttcctccaaagcctaaggacaccctgatgatctctcggacccctgaagtgacctgcgtggtggtggatgtgtctcacgaggacccagaagtgaagtttaattggtacgtggacggcgtggaagtgcacaacgccaagaccaagcctagagaggaacagtacaactccacctacagagtggtgtccgtgctgaccgtgctgcaccaggattggctgaatggcaaagagtacaagtgcaaggtgtccaacaaggccctgcctgctcctatcgaaaagaccatctccaaggctaagggccagcctcgggaacctcaggtttacacaggacctccatctcgggacgagctgacaaagaaccaggtgtccctgtcttgcgccgtgaagggcttctacccttccgacattgccgtggaatgggagtccaatggccagcctgagaacaattacaagaccacacctcctgtgctggactccgacggctcattcttcctggtgtccaagctgacagtggacaagtccagatggcagcagggcaacgtgttctcctgctctgtgatgcacgaggccctgcacaaccactacacacagaagtccctgagcctgtctcctggc

SEQ ID NO: 77 - DNA, 654 bp, synthetic construct
  source 1..654: mol_type = other DNA
gaagtgcagctgctggaatctggcggaggattggttcagcctggcggctctctgagactgtcttgtgctgcctccggcttcaccttctccagctatatcatgatgtgggtccgacaggcccctggcaaaggactggaatgggtgtcctctatctacccctctggcggcatcaccttttacgccgataccgtgaagggcagattcaccatcagccgggacaactccaagaacaccctgtacctgcagatgaactccctgagagccgaggacaccgccgtgtactactgtgctagaatcaagctgggcaccgtgaccaccgtggattattggggacagggcacactggtcaccgtgtcctctgcttctaccaagggaccctctgtgttccctctggctccttccagcaagtctacatccggtggaaccgctgctctgggctgcctggtcaaggattactttcctgagcctgtgaccgtgtcttggaactctggtgctctgacctccggcgtgcacacatttccagctgtgctgcagtcctccggcctgtactctctgtcctctgtcgtgaccgtgccttctagctctctgggcacccagacctacatctgcaacgtgaaccacaagccttccaacaccaaggtggacaagaaggtg

SEQ ID NO: 78 - DNA, 648 bp, synthetic construct
  source 1..648: mol_type = other DNA
cagtccgctctgactcagcctgcttctgtgtctggctcccctggccagtctatcaccatctcttgtaccggcacctctagcgacgtcggcggctacaattacgtgtcctggtatcagcagcaccccggcaaggctcccaagctgatgatctacgacgtgtccaacagaccctccggcgtgtccaatcggttctctggctctaagtccggcaataccgcctctctgacaatcagtggactgcaggccgaggacgaggccgactactactgttcctcctacacctcctccagcaccagagtgtttggcaccggcaccaaagtgacagtgctgggccagcctaaggccaatcctaccgtgacactgttccctccatcctccgaggaactgcaggctaacaaggctaccctcgtgtgcctgatctccgatttttaccctggcgctgtgaccgtggcttggaaggctgatggatctcctgtgaaggccggcgtggaaaccaccaagcctagcaagcagtccaacaacaaatacgccgcctcctcctacctgtctctgacccctgaacagtggaagtcccaccggtcctactcttgccaagtgacccatgagggctccaccgtggaaaagacagtggcccctaccgagtgctcc

SEQ ID NO: 79 - DNA, 657 bp, synthetic construct
  source 1..657: mol_type = other DNA
gaagtgcgactgctggaatctggcggaggactggttaagcctgagggctctctgaagctgtcttgcgtggcctctggcttcaccttctccgactacttcatgagctgggtccgacaggctcctggcaaaggactggaatgggtcgcccacatctacaccaagtcctacaactacgccacctactactccggctccgtgaagggcagattcaccatctctagggacgactctcggagcatggtgtacctgcagatgaacaacctgagaaccgaggacaccgctacctactattgcaccagagatggcagcggctacccctctctggatttttggggacagggcacccaagtgaccgtgtcctctgcttctaccaagggaccctctgtgttccctctggctccttccagcaagtctacctctggtggaaccgctgctctgggctgcctggtcaaggattactttcctgagcctgtgacagtgtcttggaactctggcgctctgacctccggcgtgcacacatttccagctgtgctgcagtcctctggcctgtactctctgtcctctgtcgtgaccgtgccttctagctctctgggcacccagacctacatctgcaacgtgaaccacaagccttccaacaccaaggtggacaagaaggtg

SEQ ID NO: 80 - DNA, 648 bp, synthetic construct
  source 1..648: mol_type = other DNA
tacgagctgactcagcctccttccgcctctgtgaatgtgggcgagacagtgaagatcacctgttccggcgaccagctgcctaagtacttcgccgattggttccaccagcggagcgaccagacaatcctgcaagtgatctacgacgacaacaagcggcccagcggcatccctgagagaatctctggatcttcctctggcaccaccgccacactgacaatcagggatgtgcgggctgaagatgagggcgactactactgcttctccggctacgtggactccgactccaagctgtatgtgtttggctccggcacacagctgacagtgcttggaggacagcccaaggccaatcctaccgtgacactgttccctccatcctccgaggaactgcaggctaacaaggctaccctcgtgtgcctgatctccgatttttaccctggcgctgtgaccgtggcttggaaggctgatggatctcctgtgaaggccggcgtggaaaccaccaagcctagcaagcagtccaacaacaaatacgccgcctcctcctacctgtctctgacccctgaacagtggaagtcccaccggtcctactcttgccaagtgacccatgagggctccaccgtggaaaagacagtggcccctaccgagtgctcc

SEQ ID NO: 81 - DNA, 654 bp, synthetic construct
  source 1..654: mol_type = other DNA
caggtgcagctggtgcagtctggcgtggaagttaagaaacctggcgcctccgtgaaggtgtcctgcaaggcttctggctacacctttaccaactactacatgtactgggtccgacaggcccctggacagggacttgaatggatgggcggcatcaacccttctaacggcggcaccaacttcaacgagaagttcaagaacagagtgaccctgaccaccgactcctctaccaccaccgcctacatggaactgaagtccctgcagttcgacgacaccgccgtgtactactgcgccagaagagactacagattcgacatgggcttcgactactggggccagggcacaacagtgaccgtgtcctctgcttctaccaagggaccctctgtgttccctctggctccttccagcaagtctacctctggtggaaccgctgctctgggctgcctggtcaaggattactttcctgagcctgtgacagtgtcctggaactctggtgctctgacctccggcgtgcacacatttccagctgtgctgcagtcctccggcctgtactctctgtcctctgtcgtgaccgtgccttctagctctctgggcacccagacctacatctgcaacgtgaaccacaagccttccaacaccaaggtggacaagaaggtg

SEQ ID NO: 82 - DNA, 651 bp, synthetic construct
  source 1..651: mol_type = other DNA
gagatcgtgctgacccagtctcctgccacattgtctctgagtcctggcgagagagctaccctgtcctgtagagcttctaagggcgtgtccacctccggctactcctacctgcattggtatcagcagaagcccggccaggctcctagactgctgatctacctggcctcttacctggaatctggcgtgcccgctagattctctggctctggatctggcaccgacttcaccctgaccatctctagcctggaacctgaggacttcgccgtgtactactgccagcactctagggacctgcctctgacctttggcggcggaacaaaggtggaaatcaagggccagcctaaggccaatcctaccgtgacactgttccctccatcctccgaggaactgcaggctaacaaggctaccctcgtgtgcctgatctctgacttttaccctggcgctgtgaccgtggcttggaaggctgatggatctcctgtgaaggccggcgtggaaaccaccaagcctagcaagcagtccaacaacaaatacgccgcctccagctatctgtctctgacccctgagcagtggaagtcccaccggtcttactcttgccaagtgacccatgagggctccaccgtggaaaagacagtggcccctaccgagtgctcc

SEQ ID NO: 83 - DNA, 396 bp, synthetic construct
  source 1..396: mol_type = other DNA
cctacctcctccagcaccaagaaaacccagctgcagttggagcatctgctgctggacctgcagatgatcctgaacggcatcaacaactacaagaaccccaagctgacccggatgctgaccttcaagttctacatgcccaagaaggccaccgagctgaaacatctgcagtgcctggaagaggaactgaagcccctggaagaagtgctgaatctggcccagtccaagaacttccacctgaggcctcgggacctgatctccaacatcaacgtgatcgtgctggaactgaaaggctccgagacaaccttcatgtgcgagtacgccgacgagacagctaccatcgtggaatttctgaaccggtggatcaccttcagccagtccatcatctctacactgacc